European Patent Application EP 4 631 357 A1, published October 15, 2025. Title: LACTOCCOCUS BACTERIAL STRAINS FOR FERMENTATION OF PLANT-BASED PREPARATION. Applicant: SAS C&DAC. The sequence listing filed with the application follows.

SEQUENCE LISTING (2 sequences)

SEQ ID NO: 1 - DNA, 1189 bp, synthetic construct
  source 1..1189: mol_type = other DNA
tgctatacatgcaagttgagcgctgaaggttggtacttgtaccaactggatgagcagcgaacgggtgagtaacgcgtggggaatctgcctttgagcgggggacaacatttggaaacgaatgctaataccgcataaaaactttaaacacaagttttaagtttgaaagatgcaattgcatcactcaaagatgatcccgcgttgtattagctagttggtgaggtaaaggctcaccaaggcgatgatacatagccgacctgagagggtgatcggccacattgggactgagacacggcccaaactcctacgggaggcagcagtagggaatcttcggcaatggacgaaagtctgaccgagcaacgccgcgtgagtgaagaaggttttcggatcgtaaaactctgttggtagagaagaacgttggtgagagtggaaagctcatcaagtgacggtaactacccagaaagggacggctaactacgtgccagcagccgcggtaatacgtaggtcccgagcgttgtccggatttattgggcgtaaagcgagcgcaggtggtttattaagtctggtgtaaaaggcagtggctcaaccattgtatgcattggaaactggtagacttgagtgcaggagaggagagtggaattccatgtgtagcggtgaaatgcgtagatatatggaggaacaccggtggcgaaagcggctctctggcctgtaactgacactgaggctcgaaagcgtggggagcaaacaggattagataccctggtagtccacgccgtaaacgatgagtgctagatgtagggagctataagttctctgtatcgcagctaacgcaataagcactccgcctggggagtacgaccgcaaggttgaaactcaaaggaattgacgggggcccgcacaagcggtggagcatgtggtttaattcgaagcaacgcgaagaaccttaccaggtcttgacatactcgtgctattcctagagataggaagttccttcgggacacgggatacaggtggtgcatggttgtcgtcagctcgtgtcgtgagatgttgggttaagtcccgcaacgagcgcaacccctattgttagttgccatcattaagttgggcactctaacgagactgccggtgataaaccggaggaaggggggatgacgtcaaatcatcatgccccttatgacctgggctaccacgt

SEQ ID NO: 2 - DNA, 1207 bp, synthetic construct
  source 1..1207: mol_type = other DNA
gcttatacatgcaagttgtagcgctgaaggttggtacttgtaccaactggatgagcagcgaacgggtgagtaacgcgtggggaatctgcctttgagcgggggacaacatttggaaacgaatgctaataccgcataaaaactttaaacacaagttttaagtttgaaagatgcaattgcatcactcaaagatgatcccgcgttgtattagctagttggtgaggtaaaggctcaccaaggcgatgatacatagccgacctgagagggtgatcggccacattgggactgagacacggcccaaactcctacgggaggcagcagtagggaatcttcggcaatggacgaaagtctgaccgagcaacgccgcgtgagtgaagaaggttttcggatcgtaaaactctgttggtagagaagaacgttggtgagagtggaaagctcatcaagtgacggtaactacccagaaagggacggctaactacgtgccagcagccgcggtaatacgtaggtcccgagcgttgtccggatttattgggcgtaaagcgagcgcaggtggtttattaagtctggtgtaaaaggcagtggctcaaccattgtatgcattggaaactggtagacttgagtgcaggagaggagagtggaattccatgtgtagcggtgaaatgcgtagatatatggaggaacaccggtggcgaaagcggctctctggcctgtaactgacactgaggctcgaaagcgtggggagcaaacaggattagataccctggtagtccacgccgtaaacgatgagtgctagatgtagggagctataagttctctgtatcgcagctaacgcaataagcactccgcctggggagtacgaccgcaaggttgaaactcaaaggaattgacgggggcccgcacaagcggtggagcatgtggtttaattcgaagcaacgcgaagaaccttaccaggtcttgacatactcgtgctattcctagagataggaagttccttcgggacacgggatacaggtggtgcatggttgtcgtcagctcgtgtcgtgagatgttgggttaagtcccgcaacgagcgcaacccctattgttagttgccatcattaagttgggcactctaacgagactgccggtgataaaccggaggaaggtggggatgacgtcaatcatcatgccccttatgacctgggctaccacgtgctacatggatggtaca